European Patent Specification EP 4 185 694 B1, published February 18, 2026. Title: Combinatorial inhibition of miRNAs for treatment of heart failure. Applicant: Goethe Universitaet. The sequence listing filed with the application follows.

SEQUENCE LISTING (26 sequences)

SEQ ID NO: 1 - DNA, 15 bp, Artificial Sequence
  miRNA inhibitors
acttctttacattcc

SEQ ID NO: 2 - DNA, 15 bp, Artificial Sequence
  miRNA inhibitors
ccatgatgtgctgct

SEQ ID NO: 3 - DNA, 16 bp, Artificial Sequence
  miRNA inhibitors
accaatcagctaagct

SEQ ID NO: 4 - DNA, 15 bp, Artificial Sequence
  miRNA inhibitors
agctaagacactgcc

SEQ ID NO: 5 - DNA, 16 bp, Artificial Sequence
  miRNA inhibitors
accattatgtgctgct

SEQ ID NO: 6 - DNA, 15 bp, Artificial Sequence
  miRNA inhibitors
tatttacgtgctgct

SEQ ID NO: 7 - DNA, 16 bp, Artificial Sequence
  miRNA inhibitors
gatttcagatggtgct

SEQ ID NO: 8 - DNA, 16 bp, Artificial Sequence
  miRNA inhibitors
agctaattacactgcc

SEQ ID NO: 9 - DNA, 16 bp, Artificial Sequence
  miRNA inhibitors
agctaactacactgcc

SEQ ID NO: 10 - DNA, 15 bp, Artificial Sequence
  miRNA inhibitors
cgggacaagtgcaat

SEQ ID NO: 11 - DNA, 16 bp, Artificial Sequence
  miRNA inhibitors
atggctgtagactgtt

SEQ ID NO: 12 - DNA, 15 bp, Artificial Sequence
  miRNA inhibitors
gttgaaggggaccaa

SEQ ID NO: 13 - DNA, 16 bp, Artificial Sequence
  miRNA inhibitors
atgctaacaggtagga

SEQ ID NO: 14 - DNA, 16 bp, Artificial Sequence
  miRNA inhibitors
atatttctgtgctgct

SEQ ID NO: 15 - DNA, 16 bp, Artificial Sequence
  miRNA inhibitors
ctttttgctcgtctta

SEQ ID NO: 16 - DNA, 16 bp, Artificial Sequence
  miRNA inhibitors
accacagtgtgctgct

SEQ ID NO: 17 - DNA, 16 bp, Artificial Sequence
  miRNA inhibitors
gactcacaagttcctg

SEQ ID NO: 18 - DNA, 16 bp, Artificial Sequence
  miRNA inhibitors
tcctagaaagagtaga

SEQ ID NO: 19 - RNA, 22 nt, Homo sapiens
uggaauguaaagaaguauguau

SEQ ID NO: 20 - RNA, 22 nt, Mus musculus
uggaauguaaagaaguauguau

SEQ ID NO: 21 - RNA, 22 nt, Homo sapiens
uagcagcacaucaugguuuaca

SEQ ID NO: 22 - RNA, 22 nt, Mus musculus
uagcagcacaucaugguuuaca

SEQ ID NO: 23 - RNA, 22 nt, Homo sapiens
agagcuuagcugauuggugaac

SEQ ID NO: 24 - RNA, 22 nt, Mus musculus
agagcuuagcugauuggugaac

SEQ ID NO: 25 - RNA, 22 nt, Homo sapiens
uggcagugucuuagcugguugu

SEQ ID NO: 26 - RNA, 22 nt, Mus musculus
uggcagugucuuagcugguugu